European Patent Application EP 4 306 133 A1, published January 17, 2024. Title: Composition for administration of double-stranded oligonucleotide structures using an ultrasonic nebulizer for prevention or treatment of respiratory viral infection including COVID-19, pulmonary fibrosis caused by viral infection, or respiratory diseases. Applicant: BIONEER CORPORATION siRNAgen Therapeutics Corporation. The sequence listing filed with the application follows.

SEQUENCE LISTING (30 sequences)

SEQ ID NO: 1 - DNA, 20 bp, Artificial Sequence
  Primer
acacctactctgggaagcgt

SEQ ID NO: 2 - DNA, 20 bp, Artificial Sequence
  Primer
gccaggtatttgtggttcgt

SEQ ID NO: 3 - DNA, 20 bp, Artificial Sequence
  Primer
ccagcaatcaagtttgccta

SEQ ID NO: 4 - DNA, 20 bp, Artificial Sequence
  Primer
gtggtggtggtggtaattca

SEQ ID NO: 5 - DNA, 19 bp, Artificial Sequence
  AREG Target Sequence
ctgggaagcgtgaaccatt

SEQ ID NO: 6 - RNA, 19 nt, Artificial Sequence
  AREG Target Sequence
aaugguucacgcuucccag

SEQ ID NO: 7 - DNA, 50 bp, Artificial Sequence
  Primer
gtcgtatccagtgcagggtccgaggtattcgcactggatacgaccggatt

SEQ ID NO: 8 - DNA, 18 bp, Artificial Sequence
  Primer
cgcatgcgcttctcttca

SEQ ID NO: 9 - DNA, 16 bp, Artificial Sequence
  Primer
gtgcagggtccgaggt

SEQ ID NO: 10 - DNA, 22 bp, Artificial Sequence
  Primer
cgcactggatacgaccggattg

SEQ ID NO: 11 - DNA, 19 bp, Artificial Sequence
  sense
aatagagctcgcaccgtag

SEQ ID NO: 12 - RNA, 19 nt, Artificial Sequence
  antisense
cuacggugcgagcucuauu

SEQ ID NO: 13 - DNA, 19 bp, Artificial Sequence
  sense
tggtactggtaagagtcat

SEQ ID NO: 14 - RNA, 19 nt, Artificial Sequence
  antisense
augacucuuaccaguacca

SEQ ID NO: 15 - DNA, 19 bp, Artificial Sequence
  sense
gtttatcacccgcgaagaa

SEQ ID NO: 16 - RNA, 19 nt, Artificial Sequence
  antisense
uucuucgcgggugauaaac

SEQ ID NO: 17 - DNA, 19 bp, Artificial Sequence
  sense
cataacagatgcgcaaaca

SEQ ID NO: 18 - RNA, 19 nt, Artificial Sequence
  antisense
uguuugcgcaucuguuaug

SEQ ID NO: 19 - DNA, 19 bp, Artificial Sequence
  sense
ataatgatgaatgtcgcaa

SEQ ID NO: 20 - RNA, 19 nt, Artificial Sequence
  antisense
uugcgacauucaucauuau

SEQ ID NO: 21 - DNA, 19 bp, Artificial Sequence
  sense
ttaaaaccaacactaccac

SEQ ID NO: 22 - RNA, 19 nt, Artificial Sequence
  antisense
gugguaguguugguuuuaa

SEQ ID NO: 23 - DNA, 19 bp, Artificial Sequence
  sense
atagtagggatgacattac

SEQ ID NO: 24 - RNA, 19 nt, Artificial Sequence
  antisense
guaaugucaucccuacuau

SEQ ID NO: 25 - DNA, 19 bp, Artificial Sequence
  sense
tctctatcagacattatgc

SEQ ID NO: 26 - RNA, 19 nt, Artificial Sequence
  antisense
gcauaaugucugauagaga

SEQ ID NO: 27 - DNA, 19 bp, Artificial Sequence
  sense
gcttcttcgcgggtgataa

SEQ ID NO: 28 - RNA, 19 nt, Artificial Sequence
  antisense
uuaucacccgcgaagaagc

SEQ ID NO: 29 - DNA, 19 bp, Artificial Sequence
  sense
ccatccgaaagggagtgag

SEQ ID NO: 30 - RNA, 19 nt, Artificial Sequence
  antisense
cucacucccuuucggaugg